European Patent Application EP 4 703 384 A1, published March 4, 2026. Title: 靶向G蛋白偶联受体的双特异性抗体. Applicant: 正大天晴药业集团股份有限公司. Application CN. The sequence listing filed with the application follows.

SEQUENCE LISTING (104 sequences)

SEQ ID NO: 1 - protein, 5 aa, synthetic construct
NYVMH

SEQ ID NO: 2 - protein, 17 aa, synthetic construct
YFNPYNDGTNYNEKFKG

SEQ ID NO: 3 - protein, 9 aa, synthetic construct
GGVRRYFDV

SEQ ID NO: 4 - protein, 11 aa, synthetic construct
RASQDIGSNLN

SEQ ID NO: 5 - protein, 7 aa, synthetic construct
ATFSLDS

SEQ ID NO: 6 - protein, 9 aa, synthetic construct
QQYANFPPT

SEQ ID NO: 7 - protein, 118 aa, synthetic construct
EVQLQQSGPELVKPGASVKMSCKASGYTFTNYVMHWVKQKPGQGLEWIGYFNPYNDGTNYNEKFKGKATLTSDKSSNTAYMELSSLTSEDSAVYYCARGGVRRYFDVWGAGTTVTVSS

SEQ ID NO: 8 - protein, 107 aa, synthetic construct
DIQMTQSPSSLSASLGERVSLTCRASQDIGSNLNWLQLGPDGTIKRLIYATFSLDSGVPKRFSGSRSGSDYSLTISSLESEDFVDYYCQQYANFPPTFGGGTKLEIK

SEQ ID NO: 9 - protein, 10 aa, synthetic construct
GFTFSNYGMS

SEQ ID NO: 10 - protein, 17 aa, synthetic construct
SISSGGGRIYYPDNVKG

SEQ ID NO: 11 - protein, 5 aa, synthetic construct
HAMDN

SEQ ID NO: 12 - protein, 10 aa, synthetic construct
SASSSVSNMY

SEQ ID NO: 13 - protein, 7 aa, synthetic construct
DTSKLAS

SEQ ID NO: 14 - protein, 9 aa, synthetic construct
QQWSSNPLT

SEQ ID NO: 15 - protein, 114 aa, synthetic construct
EVKLVESGGGLVKPGASLKLSCAASGFTFSNYGMSWVRQTSDKRLEWVASISSGGGRIYYPDNVKGRFTISRENAKNTLYLQMSSLKSEDTALYYCTRHAMDNWGQGTSVIVSS

SEQ ID NO: 16 - protein, 106 aa, synthetic construct
QIVLTQSPAIMSASPGEKVTMTCSASSSVSNMYWYQQKSGTSPKRWIYDTSKLASGVPARFSGSGSGTSYSLTISSMEAEDASTYYCQQWSSNPLTFGAGTTLELK

SEQ ID NO: 17 - protein, 10 aa, synthetic construct
GFTFSSYGMS

SEQ ID NO: 18 - protein, 17 aa, synthetic construct
TISSGGSYTYYPDSVKG

SEQ ID NO: 19 - protein, 9 aa, synthetic construct
QALRYHMDS

SEQ ID NO: 20 - protein, 11 aa, synthetic construct
KASQNVGTNVA

SEQ ID NO: 21 - protein, 7 aa, synthetic construct
SASYRYS

SEQ ID NO: 22 - protein, 9 aa, synthetic construct
QQYYSYPWT

SEQ ID NO: 23 - protein, 118 aa, synthetic construct
EVQLVESGGDLVKPGGSLKLSCAASGFTFSSYGMSWVRQTPDKRLEWVATISSGGSYTYYPDSVKGRFTFSRDNAKNTLYLQMSSLKSEDTAMYYCVRQALRYHMDSWGQGTSVTVSS

SEQ ID NO: 24 - protein, 107 aa, synthetic construct
DIVMTQSQKFMSTSVGDRVSVTCKASQNVGTNVAWYQQKPGQSPKALIYSASYRYSGVPDRFTGSGSGTDFTLTISNVQSEDLADFFCQQYYSYPWTFGGGTKLEIK

SEQ ID NO: 25 - protein, 10 aa, synthetic construct
GYTFTDYYMN

SEQ ID NO: 26 - protein, 17 aa, synthetic construct
YIYPNNGGTGYNQRFKG

SEQ ID NO: 27 - protein, 13 aa, synthetic construct
WGGTRLGYYAMDY

SEQ ID NO: 28 - protein, 11 aa, synthetic construct
KASQNVGTNVV

SEQ ID NO: 29 - protein, 7 aa, synthetic construct
WASTRHT

SEQ ID NO: 30 - protein, 9 aa, synthetic construct
QQYSRYPYT

SEQ ID NO: 31 - protein, 122 aa, synthetic construct
EVQLQQSGPELVKPGASVKMSCKASGYTFTDYYMNWVKQSHGKSLEWIGYIYPNNGGTGYNQRFKGKATLTADKSSSTAYMELRSLTSEDSAVYYCARWGGTRLGYYAMDYWGQGTSVTVSS

SEQ ID NO: 32 - protein, 107 aa, synthetic construct
DIVMTQSQKFMSTSVGDRVSVTCKASQNVGTNVVWYQQKPGQSPKLLIYWASTRHTGVPDRFTGSGSGTDFTLTISNVQSEDLADYFCQQYSRYPYTFGGGTKLEIK

SEQ ID NO: 33 - protein, 5 aa, synthetic construct
SFGMH

SEQ ID NO: 34 - protein, 17 aa, synthetic construct
YISRGSSTIYYADTVKG

SEQ ID NO: 35 - protein, 12 aa, synthetic construct
SGYGSSSYYFDY

SEQ ID NO: 36 - protein, 12 aa, synthetic construct
RASSSIRSSYLH

SEQ ID NO: 37 - protein, 7 aa, synthetic construct
STSNLAS

SEQ ID NO: 38 - protein, 9 aa, synthetic construct
QQFSGYPLT

SEQ ID NO: 39 - protein, 121 aa, synthetic construct
DVQLVESGGGLVQPGGSRKVSCAASGFTFSSFGMHWVRQAPEKGLEWVAYISRGSSTIYYADTVKGRFTISRDNPKNTLFLQMTSLRSEDTAMYYCARSGYGSSSYYFDYWGQGTTLTVSS

SEQ ID NO: 40 - protein, 108 aa, synthetic construct
ENVLTQSPAIMSASPREKVTMTCRASSSIRSSYLHWYQQKSGASPKLWIYSTSNLASGVPARFSGSGSGTSYSLTISSVEAEDAATYYCQQFSGYPLTFGGGTKLEIK

SEQ ID NO: 41 - protein, 345 aa, synthetic construct
MYKDCIESTGDYFLLCDAEGPWGIILESLAILGIVVTILLLLAFLFLMRKIQDCSQWNVLPTQLLFLLSVLGLFGLAFAFIIELNQQTAPVRYFLFGVLFALCFSCLLAHASNLVKLVRGCVSFSWTTILCIAIGCSLLQIIIATEYVTLIMTRGMMFVNMTPCQLNVDFVVLLVYVLFLMALTFFVSKATFCGPCENWKQHGRLIFITVLFSIIIWVVWISMLLRGNPQFQRQPQWDDPVVCIALVTNAWVFLLLYIVPELCILYRSCRQECPLQGNACPVTAYQHSFQVENQELSRARDSDGAEEDVALTSYGTPIQPQTVDPTQECFIPQAKLSPQQDAGGV

SEQ ID NO: 42 - protein, 344 aa, synthetic construct
MYKDCIESTGDYFLPCDSEGPWGIILESLAILGIVVTILLLLAFLFLMRKIQDCSQWNVLPTQLLFLLSVLGLFGLAFAFIIQLNQQTAPVRYFLFGVLFALCFSCLLAHASNLVKLVRGRVSFSWTTILCIAIGCSLLQVIIAIEYVTLIMTRGMMFVHMTPYQLNVDFVVLLVYVLFLMALTFFVSKATFCGPCENWKQHGRLIFITVLFSIIIWVVWISMLLRGNPQFQRQPQWDDPVVCIALVTNAWVFLLLYIVPELCILYRSCRQECPSQGHACPVTAYQRSFQVENQELSRARDSDGAEEDVALTSFGTPIQPQTVDPTQECFIPRAKLSPQQDAGV

SEQ ID NO: 43 - protein, 344 aa, synthetic construct
MYEDCVKSTEDYYLFCDNEGPWAIVLESLAVIGIVVTILLLLAFLFLMRKVQDCSQWNVLPTQFLFLLAVLGLFGLTFAFIIQLNHQTAPVRYFLFGVLFAICFSCLLAHASNLVKLVRGRVSFCWTTILFIAIGVSLLQTIIAIEYVTLIMTRGLMFEHMTPYQLNVDFVCLLIYVLFLMALTFFVSKATFCGPCENWKQHGRLIFATVLVSIIIWVVWISMLLRGNPQLQRQPHWDDAVICIGLVTNAWVFLLIYIIPELSILYRSCRQECPTQGNVCQVPVYQRSFRMDTQEPTRARDSDGAQEDVALTAYGTPIQLQSADPSREYLIPSATLSPQQDAGL

SEQ ID NO: 44 - protein, 118 aa, synthetic construct
QVQLVQSGAEVKKPGASVKVSCKASGYSFTGYTMNWVRQAPGQGLEWMGLINPYNSDTNYAQKLQGRVTMTTDTSTSTAYMELRSLRSDDTAVYYCARVALRVALDYWGQGTLVTVSS

SEQ ID NO: 45 - protein, 107 aa, synthetic construct
DIQMTQSPSSLSASVGDRVTITCKASQNVATHVGWYQQKPGKAPKRLIYSASYRYSGVPSRFSGSGSGTEFTLTISNLQPEDFATYYCQQYNRYPYTFGQGTKLEIK

SEQ ID NO: 46 - protein, 357 aa, synthetic construct
MATTVPDGCRNGLKSKYYRLCDKAEAWGIVLETVATAGVVTSVAFMLTLPILVCKVQDSNRRKMLPTQFLFLLGVLGIFGLTFAFIIGLDGSTGPTRFFLFGILFSICFSCLLAHAVSLTKLVRGRKPLSLLVILGLAVGFSLVQDVIAIEYIVLTMNRTNVNVFSELSAPRRNEDFVLLLTYVLFLMALTFLMSSFTFCGSFTGWKRHGAHIYLTMLLSIAIWVAWITLLMLPDFDRRWDDTILSSALAANGWVFLLAYVSPEFWLLTKQRNPMDYPVEDAFCKPQLVKKSYGVENRAYSQEEITQGFEETGDTLYAPYSTHFQLQNQPPQKEFSIPRAHAWPSPYKDYEVKKEGS

SEQ ID NO: 47 - protein, 403 aa, synthetic construct
MFVASERKMRAHQVLTFLLLFVITSVASENASTSRGCGLDLLPQYVSLCDLDAIWGIVVEAVAGAGALITLLLMLILLVRLPFIKEKEKKSPVGLHFLFLLGTLGLFGLTFAFIIQEDETICSVRRFLWGVLFALCFSCLLSQAWRVRRLVRHGTGPAGWQLVGLALCLMLVQVIIAVEWLVLTVLRDTRPACAYEPMDFVMALIYDMVLLVVTLGLALFTLCGKFKRWKLNGAFLLITAFLSVLIWVAWMTMYLFGNVKLQQGDAWNDPTLAITLAASGWVFVIFHAIPEIHCTLLPALQENTPNYFDTSQPRMRETAFEEDVQLPRAYMENKAFSMDEHNAALRTAGFPNGSLGKRPSGSLGKRPSAPFRSNVYQPTEMAVVLNGGTIPTAPPSHTGRHLW

SEQ ID NO: 48 - protein, 441 aa, synthetic construct
MAIHKALVMCLGLPLFLFPGAWAQGHVPPGCSQGLNPLYYNLCDRSGAWGIVLEAVAGAGIVTTFVLTIILVASLPFVQDTKKRSLLGTQVFFLLGTLGLFCLVFACVVKPDFSTCASRRFLFGVLFAICFSCLAAHVFALNFLARKNHGPRGWVIFTVALLLTLVEVIINTEWLIITLVRGSGEGGPQGNSSAGWAVASPCAIANMDFVMALIYVMLLLLGAFLGAWPALCGRYKRWRKHGVFVLLTTATSVAIWVVWIVMYTYGNKQHNSPTWDDPTLAIALAANAWAFVLFYVIPEVSQVTKSSPEQSYQGDMYPTRGVGYETILKEQKGQSMFVENKAFSMDEPVAAKRPVSPYSGYNGQLLTSVYQPTEMALMHKVPSEGAYDIILPRATANSQVMGSANSTLRAEDMYSAQSHQAATPPKDGKNSQVFRNPYVWD

SEQ ID NO: 49 - protein, 448 aa, synthetic construct
EVQLQQSGPELVKPGASVKMSCKASGYTFTNYVMHWVKQKPGQGLEWIGYFNPYNDGTNYNEKFKGKATLTSDKSSNTAYMELSSLTSEDSAVYYCARGGVRRYFDVWGAGTTVTVSSASTKGPSVFPLAPSSKSTSGGTAALGCLVKDYFPEPVTVSWNSGALTSGVHTFPAVLQSSGLYSLSSVVTVPSSSLGTQTYICNVNHKPSNTKVDKKVEPKSCDKTHTCPPCPAPELLGGPSVFLFPPKPKDTLMISRTPEVTCVVVDVSHEDPEVKFNWYVDGVEVHNAKTKPREEQYNSTYRVVSVLTVLHQDWLNGKEYKCKVSNKALPAPIEKTISKAKGQPREPQVYTLPPSRDELTKNQVSLTCLVKGFYPSDIAVEWESNGQPENNYKTTPPVLDSDGSFFLYSKLTVDKSRWQQGNVFSCSVMHEALHNHYTQKSLSLSPGK

SEQ ID NO: 50 - protein, 214 aa, synthetic construct
DIQMTQSPSSLSASLGERVSLTCRASQDIGSNLNWLQLGPDGTIKRLIYATFSLDSGVPKRFSGSRSGSDYSLTISSLESEDFVDYYCQQYANFPPTFGGGTKLEIKRTVAAPSVFIFPPSDEQLKSGTASVVCLLNNFYPREAKVQWKVDNALQSGNSQESVTEQDSKDSTYSLSSTLTLSKADYEKHKVYACEVTHQGLSSPVTKSFNRGEC

SEQ ID NO: 51 - protein, 444 aa, synthetic construct
EVKLVESGGGLVKPGASLKLSCAASGFTFSNYGMSWVRQTSDKRLEWVASISSGGGRIYYPDNVKGRFTISRENAKNTLYLQMSSLKSEDTALYYCTRHAMDNWGQGTSVIVSSASTKGPSVFPLAPSSKSTSGGTAALGCLVKDYFPEPVTVSWNSGALTSGVHTFPAVLQSSGLYSLSSVVTVPSSSLGTQTYICNVNHKPSNTKVDKKVEPKSCDKTHTCPPCPAPELLGGPSVFLFPPKPKDTLMISRTPEVTCVVVDVSHEDPEVKFNWYVDGVEVHNAKTKPREEQYNSTYRVVSVLTVLHQDWLNGKEYKCKVSNKALPAPIEKTISKAKGQPREPQVYTLPPSRDELTKNQVSLTCLVKGFYPSDIAVEWESNGQPENNYKTTPPVLDSDGSFFLYSKLTVDKSRWQQGNVFSCSVMHEALHNHYTQKSLSLSPGK

SEQ ID NO: 52 - protein, 213 aa, synthetic construct
QIVLTQSPAIMSASPGEKVTMTCSASSSVSNMYWYQQKSGTSPKRWIYDTSKLASGVPARFSGSGSGTSYSLTISSMEAEDASTYYCQQWSSNPLTFGAGTTLELKRTVAAPSVFIFPPSDEQLKSGTASVVCLLNNFYPREAKVQWKVDNALQSGNSQESVTEQDSKDSTYSLSSTLTLSKADYEKHKVYACEVTHQGLSSPVTKSFNRGEC

SEQ ID NO: 53 - protein, 448 aa, synthetic construct
EVQLVESGGDLVKPGGSLKLSCAASGFTFSSYGMSWVRQTPDKRLEWVATISSGGSYTYYPDSVKGRFTFSRDNAKNTLYLQMSSLKSEDTAMYYCVRQALRYHMDSWGQGTSVTVSSASTKGPSVFPLAPSSKSTSGGTAALGCLVKDYFPEPVTVSWNSGALTSGVHTFPAVLQSSGLYSLSSVVTVPSSSLGTQTYICNVNHKPSNTKVDKKVEPKSCDKTHTCPPCPAPELLGGPSVFLFPPKPKDTLMISRTPEVTCVVVDVSHEDPEVKFNWYVDGVEVHNAKTKPREEQYNSTYRVVSVLTVLHQDWLNGKEYKCKVSNKALPAPIEKTISKAKGQPREPQVYTLPPSRDELTKNQVSLTCLVKGFYPSDIAVEWESNGQPENNYKTTPPVLDSDGSFFLYSKLTVDKSRWQQGNVFSCSVMHEALHNHYTQKSLSLSPGK

SEQ ID NO: 54 - protein, 214 aa, synthetic construct
DIVMTQSQKFMSTSVGDRVSVTCKASQNVGTNVAWYQQKPGQSPKALIYSASYRYSGVPDRFTGSGSGTDFTLTISNVQSEDLADFFCQQYYSYPWTFGGGTKLEIKRTVAAPSVFIFPPSDEQLKSGTASVVCLLNNFYPREAKVQWKVDNALQSGNSQESVTEQDSKDSTYSLSSTLTLSKADYEKHKVYACEVTHQGLSSPVTKSFNRGEC

SEQ ID NO: 55 - protein, 452 aa, synthetic construct
EVQLQQSGPELVKPGASVKMSCKASGYTFTDYYMNWVKQSHGKSLEWIGYIYPNNGGTGYNQRFKGKATLTADKSSSTAYMELRSLTSEDSAVYYCARWGGTRLGYYAMDYWGQGTSVTVSSASTKGPSVFPLAPSSKSTSGGTAALGCLVKDYFPEPVTVSWNSGALTSGVHTFPAVLQSSGLYSLSSVVTVPSSSLGTQTYICNVNHKPSNTKVDKKVEPKSCDKTHTCPPCPAPELLGGPSVFLFPPKPKDTLMISRTPEVTCVVVDVSHEDPEVKFNWYVDGVEVHNAKTKPREEQYNSTYRVVSVLTVLHQDWLNGKEYKCKVSNKALPAPIEKTISKAKGQPREPQVYTLPPSRDELTKNQVSLTCLVKGFYPSDIAVEWESNGQPENNYKTTPPVLDSDGSFFLYSKLTVDKSRWQQGNVFSCSVMHEALHNHYTQKSLSLSPGK

SEQ ID NO: 56 - protein, 214 aa, synthetic construct
DIVMTQSQKFMSTSVGDRVSVTCKASQNVGTNVVWYQQKPGQSPKLLIYWASTRHTGVPDRFTGSGSGTDFTLTISNVQSEDLADYFCQQYSRYPYTFGGGTKLEIKRTVAAPSVFIFPPSDEQLKSGTASVVCLLNNFYPREAKVQWKVDNALQSGNSQESVTEQDSKDSTYSLSSTLTLSKADYEKHKVYACEVTHQGLSSPVTKSFNRGEC

SEQ ID NO: 57 - protein, 451 aa, synthetic construct
DVQLVESGGGLVQPGGSRKVSCAASGFTFSSFGMHWVRQAPEKGLEWVAYISRGSSTIYYADTVKGRFTISRDNPKNTLFLQMTSLRSEDTAMYYCARSGYGSSSYYFDYWGQGTTLTVSSASTKGPSVFPLAPSSKSTSGGTAALGCLVKDYFPEPVTVSWNSGALTSGVHTFPAVLQSSGLYSLSSVVTVPSSSLGTQTYICNVNHKPSNTKVDKKVEPKSCDKTHTCPPCPAPELLGGPSVFLFPPKPKDTLMISRTPEVTCVVVDVSHEDPEVKFNWYVDGVEVHNAKTKPREEQYNSTYRVVSVLTVLHQDWLNGKEYKCKVSNKALPAPIEKTISKAKGQPREPQVYTLPPSRDELTKNQVSLTCLVKGFYPSDIAVEWESNGQPENNYKTTPPVLDSDGSFFLYSKLTVDKSRWQQGNVFSCSVMHEALHNHYTQKSLSLSPGK

SEQ ID NO: 58 - protein, 215 aa, synthetic construct
ENVLTQSPAIMSASPREKVTMTCRASSSIRSSYLHWYQQKSGASPKLWIYSTSNLASGVPARFSGSGSGTSYSLTISSVEAEDAATYYCQQFSGYPLTFGGGTKLEIKRTVAAPSVFIFPPSDEQLKSGTASVVCLLNNFYPREAKVQWKVDNALQSGNSQESVTEQDSKDSTYSLSSTLTLSKADYEKHKVYACEVTHQGLSSPVTKSFNRGEC

SEQ ID NO: 59 - protein, 17 aa, synthetic construct
  SITE 7: note = D or E
  SITE 8: note = G or A
YFNPYNXXTNYNEKFKG

SEQ ID NO: 60 - protein, 17 aa, synthetic construct
YFNPYNDATNYNEKFKG

SEQ ID NO: 61 - protein, 17 aa, synthetic construct
YFNPYNEGTNYNEKFKG

SEQ ID NO: 62 - protein, 118 aa, synthetic construct
EVQLVQSGAEVVKPGASVKMSCKASGYTFTNYVMHWVKQAPGQGLEWMGYFNPYNDGTNYNEKFKGRVTLTSDTSANTAYMELSSLRSEDTAVYYCARGGVRRYFDVWGQGTTVTVSS

SEQ ID NO: 63 - protein, 118 aa, synthetic construct
EVQLVQSGAEVVKPGASVKMSCKASGYTFTNYVMHWVKQAPGQGLEWIGYFNPYNDGTNYNEKFKGRATLTSDTSANTAYMELSSLRSEDTAVYYCARGGVRRYFDVWGQGTTVTVSS

SEQ ID NO: 64 - protein, 118 aa, synthetic construct
EVQLVQSGAEVVKPGASVKMSCKASGYTFTNYVMHWVKQAPGQGLEWIGYFNPYNDATNYNEKFKGRATLTSDTSANTAYMELSSLRSEDTAVYYCARGGVRRYFDVWGQGTTVTVSS

SEQ ID NO: 65 - protein, 118 aa, synthetic construct
EVQLVQSGAEVVKPGASVKMSCKASGYTFTNYVMHWVKQAPGQGLEWIGYFNPYNEGTNYNEKFKGRATLTSDTSANTAYMELSSLRSEDTAVYYCARGGVRRYFDVWGQGTTVTVSS

SEQ ID NO: 66 - protein, 118 aa, synthetic construct
  SITE 5: note = Q or V
  SITE 9: note = P or A
  SITE 11: note = L or V
  SITE 40: note = K or A
  SITE 48: note = I or M
  SITE 56: note = D or E
  SITE 57: note = G or A
  SITE 67: note = K or R
  SITE 68: note = A or V
  SITE 74: note = K or T
  SITE 76: note = S or A
  SITE 87: note = T or R
  SITE 91: note = S or T
  SITE 110: note = A or Q
EVQLXQSGXEXVKPGASVKMSCKASGYTFTNYVMHWVKQXPGQGLEWXGYFNPYNXXTNYNEKFKGXXTLTSDXSXNTAYMELSSLXSEDXAVYYCARGGVRRYFDVWGXGTTVTVSS

SEQ ID NO: 67 - protein, 107 aa, synthetic construct
DIQMTQSPSSLSASVGDRVTITCRASQDIGSNLNWLQLGPGGAIKRLIYATFSLDSGVPSRFSGSRSGSDYTLTISSLQPEDFVDYYCQQYANFPPTFGGGTKVEIK

SEQ ID NO: 68 - protein, 121 aa, synthetic construct
EVQLVESGGGLVQPGGSRRVSCAASGFTFSSFGMHWVRQAPGKGLEWVAYISRGSSTIYYADTVKGRFTISRDNAKNSLYLQMNSLRAEDTAVYYCARSGYGSSSYYFDYWGQGTTVTVSS

SEQ ID NO: 69 - protein, 108 aa, synthetic construct
EIVLTQSPATLSASPGERATMSCRASSSIRSSYLHWYQQKPGQSPRLWIYSTSNLASGVPARFSGSGSGTDYTLTISSLEPEDAAVYYCQQFSGYPLTFGGGTKVEIK

SEQ ID NO: 70 - protein, 448 aa, synthetic construct
EVQLVQSGAEVVKPGASVKMSCKASGYTFTNYVMHWVKQAPGQGLEWMGYFNPYNDGTNYNEKFKGRVTLTSDTSANTAYMELSSLRSEDTAVYYCARGGVRRYFDVWGQGTTVTVSSASTKGPSVFPLAPSSKSTSGGTAALGCLVKDYFPEPVTVSWNSGALTSGVHTFPAVLQSSGLYSLSSVVTVPSSSLGTQTYICNVNHKPSNTKVDKKVEPKSCDKTHTCPPCPAPELLGGPSVFLFPPKPKDTLMISRTPEVTCVVVDVSHEDPEVKFNWYVDGVEVHNAKTKPREEQYNSTYRVVSVLTVLHQDWLNGKEYKCKVSNKALPAPIEKTISKAKGQPREPQVYTLPPSRDELTKNQVSLTCLVKGFYPSDIAVEWESNGQPENNYKTTPPVLDSDGSFFLYSKLTVDKSRWQQGNVFSCSVMHEALHNHYTQKSLSLSPGK

SEQ ID NO: 71 - DNA, 1344 bp, synthetic construct
  source 1..1344: mol_type = other DNA
gaagtgcagctggtgcagtctggcgccgaggtggtgaaacctggcgcctctgtcaagatgtcctgcaaggcctccggctacacattcaccaactatgtgatgcactgggtcaagcaggctcccgggcagggactggaatggatgggctacttcaacccttacaacgacggcaccaattataacgagaagttcaagggcagagtgaccctgacatctgatacctccgccaacaccgcctacatggaactgtccagcctgagatccgaggacaccgccgtgtactactgcgccagaggcggagtgcggagatacttcgacgtgtggggccaaggcaccaccgtgaccgtgtcctctgccagcaccaagggcccatccgtgtttcctctggctccttcctccaaatctaccagcggaggcaccgctgctttgggatgcctggtgaaggactactttccagagcccgtgaccgtgtcttggaacagcggcgccctgacctctggcgtgcataccttccctgctgttctgcagtccagcggcctgtactctctgtcctctgtggtgacagtgccctctagctctctgggcacccagacctacatctgcaacgtgaaccacaagccttctaataccaaagtggacaagaaggtggaacccaagtcttgcgacaagacccacacctgtcctccttgccctgctcctgaactgctgggcggcccttctgtgtttctgttccccccaaagcctaaggatacactgatgatctctcggacacctgaggtcacatgtgtggtcgtggatgtgtctcacgaggatcctgaagtgaagttcaactggtacgtggatggcgtggaagtgcacaacgccaagaccaagcctagagaggaacagtacaactccacttaccgggtagttagcgtgctgaccgtgctgcaccaggactggctgaacggcaaagagtacaagtgcaaggtgtccaacaaggctctgcctgctcctatcgagaaaaccatctcgaaggccaagggccagcctcgcgagcctcaggtgtacaccctgccccccagccgggacgagctgaccaagaaccaggtcagcctgacctgtctggtcaaaggcttctacccttccgacatcgccgtggagtgggagtccaacggtcaacctgagaacaactacaagacaacccctcctgtgctcgactccgacggctccttcttcctgtattccaagctgaccgtggacaagtccagatggcagcagggcaacgtgttctcctgctccgtgatgcacgaggccctgcataatcactacacccagaagtccctctccctgtctccaggcaag

SEQ ID NO: 72 - protein, 448 aa, synthetic construct
EVQLVQSGAEVVKPGASVKMSCKASGYTFTNYVMHWVKQAPGQGLEWIGYFNPYNDGTNYNEKFKGRATLTSDTSANTAYMELSSLRSEDTAVYYCARGGVRRYFDVWGQGTTVTVSSASTKGPSVFPLAPSSKSTSGGTAALGCLVKDYFPEPVTVSWNSGALTSGVHTFPAVLQSSGLYSLSSVVTVPSSSLGTQTYICNVNHKPSNTKVDKKVEPKSCDKTHTCPPCPAPELLGGPSVFLFPPKPKDTLMISRTPEVTCVVVDVSHEDPEVKFNWYVDGVEVHNAKTKPREEQYNSTYRVVSVLTVLHQDWLNGKEYKCKVSNKALPAPIEKTISKAKGQPREPQVYTLPPSRDELTKNQVSLTCLVKGFYPSDIAVEWESNGQPENNYKTTPPVLDSDGSFFLYSKLTVDKSRWQQGNVFSCSVMHEALHNHYTQKSLSLSPGK

SEQ ID NO: 73 - DNA, 1344 bp, synthetic construct
  source 1..1344: mol_type = other DNA
gaggtgcagctggtgcagagcggagccgaggtcgtgaaacctggcgcctctgtgaagatgtcgtgcaaggcttctggctacaccttcacgaactatgtgatgcactgggtcaagcaggctcctggccaaggactcgaatggatcggctattttaatccttacaacgacggtaccaactacaacgagaagttcaagggcagagctaccctgacctccgatacatctgccaacacagcctacatggaactcagctccttgcgctctgaggataccgctgtttactactgcgccagaggcggggtccggcggtacttcgacgtgtggggccagggcaccaccgtgacggtttcttctgcctccacaaagggcccctccgtgttccccctggccccatcctccaaatccacatccggcggaaccgctgctctgggctgcctggtgaaggactactttcctgagcctgtgacagtgtcttggaactctggcgccctgacctctggcgtgcatactttccctgccgtgctgcagtcttctggcctgtactccctgtcctctgttgtgaccgtgccaagctcctctctgggcacccagacctacatctgcaacgtgaaccacaagcctagcaacaccaaagtggacaagaaggtggaacccaagtcctgcgacaagacccacacctgtcctccttgtcccgcacccgagctgctgggcggcccttctgtgtttctgttccctcccaagcctaaggacaccctgatgatcagcagaacccccgaagtgacctgcgtagtggtggatgtgtctcacgaagaccctgaagtgaagttcaactggtacgtggatggcgtcgaggtgcacaacgccaagaccaaacctcgggaagagcagtacaacagcacatatagagtggtctccgtgctgacagtgctgcatcaggactggctgaacggcaaggagtacaagtgcaaggtgtccaacaaggccctgcctgctcctatcgagaagaccatctccaaggccaaaggccagcctagagagccccaagtgtacaccctgcctccatctcgggacgagctgaccaagaaccaggtgtccctgacctgtctggtgaagggcttctaccctagcgacatcgccgtcgaatgggagtctaatggacagcctgagaacaactacaagaccacccctcctgtgctggactccgacggctccttcttcctgtactccaagctgaccgtggataagagtagatggcagcagggcaacgtgttctcctgctccgtgatgcacgaggctctgcacaatcactacacccagaagtccctgtccctgagcccaggaaaa

SEQ ID NO: 74 - protein, 448 aa, synthetic construct
EVQLVQSGAEVVKPGASVKMSCKASGYTFTNYVMHWVKQAPGQGLEWIGYFNPYNDATNYNEKFKGRATLTSDTSANTAYMELSSLRSEDTAVYYCARGGVRRYFDVWGQGTTVTVSSASTKGPSVFPLAPSSKSTSGGTAALGCLVKDYFPEPVTVSWNSGALTSGVHTFPAVLQSSGLYSLSSVVTVPSSSLGTQTYICNVNHKPSNTKVDKKVEPKSCDKTHTCPPCPAPELLGGPSVFLFPPKPKDTLMISRTPEVTCVVVDVSHEDPEVKFNWYVDGVEVHNAKTKPREEQYNSTYRVVSVLTVLHQDWLNGKEYKCKVSNKALPAPIEKTISKAKGQPREPQVYTLPPSRDELTKNQVSLTCLVKGFYPSDIAVEWESNGQPENNYKTTPPVLDSDGSFFLYSKLTVDKSRWQQGNVFSCSVMHEALHNHYTQKSLSLSPGK

SEQ ID NO: 75 - DNA, 1344 bp, synthetic construct
  source 1..1344: mol_type = other DNA
gaagtgcagctggtgcagtctggtgccgaggtggtcaaacccggcgcctccgtgaagatgtcctgcaaggcttctggatataccttcaccaactatgtgatgcactgggtgaagcaggcccctggccagggcctggaatggatcggctactttaatccttacaacgacgccaccaactacaacgagaagttcaagggcagagctacgctgacctccgacaccagcgccaacaccgcctacatggaactgtccagcctgcggtccgaggataccgctgtgtactactgcgccagaggcggagtgcggagatacttcgacgtgtggggccaaggcaccaccgtgaccgtgtcctctgcctctaccaagggaccttctgtcttccctctggctccatcttctaagtccaccagcggcggcacagctgctctgggctgcctggtgaaagactacttccctgaacccgtgaccgtctcttggaactctggcgctctgacatctggagttcatacctttcctgccgtgctgcagtcctccggcctgtactccctgtcttccgtcgtgacagtgcccagcagcagcctgggcacccagacctacatctgcaacgtgaaccacaagccttccaacaccaaagtggacaagaaggtggaacctaagtcttgcgacaagacccacacctgtcctccttgtcctgctcctgagctgctgggaggccctagcgtgtttctgttcccccccaagcctaaggacaccctgatgatctcccggacacctgaagtgacctgcgtggtggtggatgtgtctcacgaggatcccgaggtgaagttcaactggtacgtggacggcgtggaagtgcacaacgccaagaccaagccccgcgaggaacagtacaactcgacatacagagtggtgtctgtgctcacagtactgcaccaggactggctgaacggcaaagagtacaagtgcaaggtctccaacaaggccctgccagctcctatcgagaaaaccatctccaaggccaaaggccagcccagagagccccaagtgtacacactgcctccaagccgggacgagctgaccaagaaccaggtgtccctgacctgtctggtcaagggcttctatccttctgacatcgccgtggagtgggagtccaatggccagcctgagaacaactacaagacaacccctcctgtgctggactccgatggctccttcttcctctactcaaagctgaccgtggataagtccagatggcagcagggcaacgtgttctcctgctccgtgatgcacgaggccctgcataatcactacacccagaagtctctgtccctctctcctggcaag

SEQ ID NO: 76 - protein, 448 aa, synthetic construct
EVQLVQSGAEVVKPGASVKMSCKASGYTFTNYVMHWVKQAPGQGLEWIGYFNPYNEGTNYNEKFKGRATLTSDTSANTAYMELSSLRSEDTAVYYCARGGVRRYFDVWGQGTTVTVSSASTKGPSVFPLAPSSKSTSGGTAALGCLVKDYFPEPVTVSWNSGALTSGVHTFPAVLQSSGLYSLSSVVTVPSSSLGTQTYICNVNHKPSNTKVDKKVEPKSCDKTHTCPPCPAPELLGGPSVFLFPPKPKDTLMISRTPEVTCVVVDVSHEDPEVKFNWYVDGVEVHNAKTKPREEQYNSTYRVVSVLTVLHQDWLNGKEYKCKVSNKALPAPIEKTISKAKGQPREPQVYTLPPSRDELTKNQVSLTCLVKGFYPSDIAVEWESNGQPENNYKTTPPVLDSDGSFFLYSKLTVDKSRWQQGNVFSCSVMHEALHNHYTQKSLSLSPGK

SEQ ID NO: 77 - DNA, 1344 bp, synthetic construct
  source 1..1344: mol_type = other DNA
gaggtgcagctggtgcagtccggcgccgaggttgtgaagcctggagcctccgtgaagatgtcctgcaaggcctccggctacaccttcaccaactacgtgatgcactgggtgaagcaggcccctggccaaggcctggaatggatcggctatttcaacccttacaacgagggcaccaactataatgaaaagttcaagggcagagccaccctgacctccgacacatctgccaacaccgcctacatggaactgtcctccctgagatctgaggatacagccgtgtactactgcgccagaggcggcgtgcggcggtacttcgacgtgtggggccagggcacaaccgtgaccgtgtcttctgcttctaccaagggcccttccgtgttccctctggctccctcttccaagtccacctccggcggcaccgctgctctcggctgtctggtgaaggattactttcctgaacccgtgacggtgtcctggaacagcggcgctctgacctctggtgtgcatacatttccagctgtgctgcagtcctctggactgtactctttgtcttctgtggtcaccgtgcctagcagctctctgggcacccagacctacatctgcaacgtgaaccacaagccttccaacaccaaagtggacaagaaggtggagcccaaatcttgcgacaaaacccacacctgtcctccttgccctgcacctgagctgctgggcggaccaagcgtctttctgttcccacctaagcccaaggataccctgatgatctcccggaccccagaagtgacctgtgtggtggtggatgtgtctcacgaggaccctgaggtcaagttcaactggtacgtggacggagtggaagtgcacaacgccaagaccaagcccagagaggaacagtacaactccacctacagagtggtgtccgttctgaccgtgctgcaccaggactggctgaacggtaaagagtacaagtgcaaggtgtccaacaaggccctgcctgctcctatcgagaagaccatctctaaggctaagggccagcctcgcgagcctcaagtatacacactgcctccctctcgggacgagctgaccaagaaccaggtgtccctgacctgcctggtcaaaggcttctacccctccgacatcgccgtcgaatgggagagtaatggacagcccgagaacaactacaagaccacccctcctgtgctggactccgacggcagcttcttcctgtactccaagctgacagtggataaatctagatggcagcagggcaacgtgttctcctgcagcgtgatgcacgaggccctgcacaatcattacacccagaagagcttgtccctgtctcctggcaag

SEQ ID NO: 78 - protein, 214 aa, synthetic construct
DIQMTQSPSSLSASVGDRVTITCRASQDIGSNLNWLQLGPGGAIKRLIYATFSLDSGVPSRFSGSRSGSDYTLTISSLQPEDFVDYYCQQYANFPPTFGGGTKVEIKRTVAAPSVFIFPPSDEQLKSGTASVVCLLNNFYPREAKVQWKVDNALQSGNSQESVTEQDSKDSTYSLSSTLTLSKADYEKHKVYACEVTHQGLSSPVTKSFNRGEC

SEQ ID NO: 79 - DNA, 642 bp, synthetic construct
  source 1..642: mol_type = other DNA
gatatccagatgacccagtccccctccagtctgtctgcttccgtgggcgacagagtgaccatcacctgtcgcgccagccaggacatcggctccaacctgaactggctgcagctgggccctggcggcgctatcaagcggctgatctatgctacatttagcctggactccggcgttccttccagattctccggctctcggtccggatctgactacaccctgacgatctccagcctgcagcctgaggacttcgtggattactactgccagcagtacgccaattttcctcctaccttcggcggaggcaccaaagtggaaatcaaaagaaccgtggctgctcctagcgtgttcatcttccccccatccgacgagcagctgaagtctggaacagcctctgtcgtgtgcctgctgaacaacttctacccccgggaagccaaggtgcagtggaaggtggacaacgccctgcagtctggcaactcccaagagtccgtcaccgagcaagattctaaggactctacctactctctcagctctaccctgacactgtccaaggccgactacgagaagcacaaggtgtacgcctgcgaagtgacccaccagggcctgtcctctcctgtgaccaagtccttcaacagaggcgagtgc

SEQ ID NO: 80 - protein, 451 aa, synthetic construct
EVQLVESGGGLVQPGGSRRVSCAASGFTFSSFGMHWVRQAPGKGLEWVAYISRGSSTIYYADTVKGRFTISRDNAKNSLYLQMNSLRAEDTAVYYCARSGYGSSSYYFDYWGQGTTVTVSSASTKGPSVFPLAPSSKSTSGGTAALGCLVKDYFPEPVTVSWNSGALTSGVHTFPAVLQSSGLYSLSSVVTVPSSSLGTQTYICNVNHKPSNTKVDKKVEPKSCDKTHTCPPCPAPELLGGPSVFLFPPKPKDTLMISRTPEVTCVVVDVSHEDPEVKFNWYVDGVEVHNAKTKPREEQYNSTYRVVSVLTVLHQDWLNGKEYKCKVSNKALPAPIEKTISKAKGQPREPQVYTLPPSRDELTKNQVSLTCLVKGFYPSDIAVEWESNGQPENNYKTTPPVLDSDGSFFLYSKLTVDKSRWQQGNVFSCSVMHEALHNHYTQKSLSLSPGK

SEQ ID NO: 81 - DNA, 1353 bp, synthetic construct
  source 1..1353: mol_type = other DNA
gaggtgcagctggtcgagtccggcggtggcctcgtgcagcctggcggctctcggcgcgtgtcttgtgctgcttctggattcaccttcagctctttcggcatgcactgggtccggcaggccccaggcaagggcctggaatgggtggcctacatctctagaggctctagcaccatctactacgccgacaccgtgaaaggcagattcaccatctccagagacaacgccaagaactccctgtacctgcagatgaactccctgagagccgaggataccgccgtgtactactgcgccagatccggctacggcagctcctcctactatttcgattactggggccagggcaccaccgtgaccgtttcctccgcctctaccaagggacctagcgtgttccctctggccccctcttctaagtccacatctggcggaaccgctgctctcggctgcctggtgaaggactactttccagagcctgtgaccgtgtcctggaactctggcgctctgacctccggcgtgcatacctttcctgctgtgctgcaatcttctggcctgtactccctgtcttccgtggtgacagtgccttctagtagcctgggcacccagacctacatctgcaacgtgaaccacaagccctctaacaccaaggtggacaagaaagtggaacccaagagctgcgacaagacccacacctgccctccttgtcctgctcctgaactgctgggcggcccttctgtgtttctgttccccccaaagcctaaggatacactgatgatctctcggacccctgaagtgacctgcgtggtggtggacgtgtctcacgaggaccctgaggtgaagttcaactggtacgtggatggagtggaagtgcacaacgccaagacaaaacctcgggaagagcagtacaattccacctacagagtggtctccgtgctgactgtgctgcatcaggactggctgaacggcaaagagtacaagtgcaaggtgtccaacaaggccctgcccgctcctatcgagaagaccatctccaaggctaagggccaacctagagaacctcaggtgtacaccctgcctccttcccgggacgagctgaccaagaaccaggttagcctgacctgtctggtgaagggcttctacccttccgacatcgccgtggagtgggagtctaatggccagcctgagaacaactacaagaccacaccccccgtgctggacagcgacggcagcttcttcctgtattccaagctgacagtcgataaatccagatggcagcagggcaacgtgttctcctgctccgtgatgcacgaggccctgcacaatcactacacccagaagtctttgtctctgtccccaggaaaa

SEQ ID NO: 82 - protein, 215 aa, synthetic construct
EIVLTQSPATLSASPGERATMSCRASSSIRSSYLHWYQQKPGQSPRLWIYSTSNLASGVPARFSGSGSGTDYTLTISSLEPEDAAVYYCQQFSGYPLTFGGGTKVEIKRTVAAPSVFIFPPSDEQLKSGTASVVCLLNNFYPREAKVQWKVDNALQSGNSQESVTEQDSKDSTYSLSSTLTLSKADYEKHKVYACEVTHQGLSSPVTKSFNRGEC

SEQ ID NO: 83 - DNA, 645 bp, synthetic construct
  source 1..645: mol_type = other DNA
gagatcgtgctgacccaaagcccagctaccctgagcgccagccccggcgagagagctaccatgtcctgcagagcctccagctctatccggtcctcctacctgcactggtaccagcagaagcctggccagtcccctcggctgtggatctattccaccagcaatctcgcctctggcgtgcctgctaggttttccggctctggatcgggaaccgactacaccctgaccatctcctctctggaacccgaggatgccgccgtgtactactgccagcagttctccggctaccctctgacattcggcggaggcaccaaagtggaaatcaagagaaccgtggctgctccttctgtgttcatcttccctccttccgacgagcagctgaagtctggcaccgcttctgtcgtgtgcctgctgaacaacttctaccccagagaggccaaggtgcagtggaaggtggacaacgctctgcagtctggcaactcccaagagtctgtcacagaacaggactccaaagattctacctactctctgtcttccacactgacactgtccaaggccgactacgagaagcacaaggtttacgcctgcgaggtgacccaccagggcctgtcctctcctgtgaccaagtccttcaaccggggcgaatgt

SEQ ID NO: 84 - protein, 448 aa, synthetic construct
EVQLVQSGAEVVKPGASVKMSCKASGYTFTNYVMHWVKQAPGQGLEWMGYFNPYNDGTNYNEKFKGRVTLTSDTSANTAYMELSSLRSEDTAVYYCARGGVRRYFDVWGQGTTVTVSSASTKGPSVFPLAPSSKSTSGGTAALGCLVKDYFPEPVTVSWNSGALTSGVHTFPAVLQSSGLYSLSSVVTVPSSSLGTQTYICNVNHKPSNTKVDKKVEPKSCDKTHTCPPCPAPEAAGGPSVFLFPPKPKDTLMISRTPEVTCVVVDVSHEDPEVKFNWYVDGVEVHNAKTKPREEQYNSTYRVVSVLTVLHQDWLNGKEYKCKVSNKALAAPIEKTISKAKGQPREPQVCTLPPSREEMTKNQVSLSCAVKGFYPSDIAVEWESNGQPENNYKTTPPVLDSDGSFFLVSKLTVDKSRWQQGNVFSCSVMHEALHNHYTQKSLSLSPGK

SEQ ID NO: 85 - DNA, 1344 bp, synthetic construct
  source 1..1344: mol_type = other DNA
gaagtgcagctggtgcagtccggcgccgaggttgtgaagcctggagccagcgtcaagatgtcctgcaaggcttctggctacaccttcaccaattatgtgatgcactgggtgaagcaggcccccggccaaggcctggaatggatgggctacttcaacccttacaacgacggcaccaactacaacgagaagttcaagggcagagtgacactgacctccgacaccagcgccaacacagcctacatggaactgtcctctctgcggtccgaggataccgccgtgtactactgcgcccggggcggcgtgcggagatacttcgacgtgtggggccaaggaaccaccgtgaccgtctcctctgcctctactaagggcccttctgtgttccctctggctccttcttccaagtctacctccggcggcaccgctgccctgggctgcctggtcaaggactacttccccgaacctgtgacagtgtcttggaactctggcgctctgacatctggtgtgcatacctttcctgccgtgctgcagtcttctggactgtactccctgtctagcgtggtgaccgtgcccagcagctccctgggaacccagacctacatctgcaacgtgaaccacaagccatccaacaccaaagtggacaagaaggtcgagcccaaatcttgcgacaagacccacacctgtcctccttgtcctgctcctgaggctgctggtggaccttccgtgtttctgttcccacctaaacccaaggacaccctgatgatcagcagaacccctgaagtgacctgcgtggtggtggatgtgtctcacgaggaccccgaggtgaagttcaactggtacgtggatggcgtggaagtgcacaacgctaagaccaagcctagagaggaacagtacaactccacctatagagtcgtgtctgtgctgaccgtgctgcaccaggactggctgaacggcaaagagtacaagtgcaaggtgtccaacaaggccctggccgctcccatcgagaaaaccatctccaaagccaagggccagcctcgggagcctcaggtgtgcacgctgcctccatctcgcgaagagatgaccaagaaccaggtcagcctgagctgtgctgtgaaaggcttttacccctccgacatcgccgtggagtgggagagcaatggccagcctgagaacaactacaagaccacacctcctgtgctggactccgacggctccttcttcctggtgtccaagctgaccgtcgataagtccagatggcagcagggcaacgtgttctcctgctctgtgatgcacgaggccctgcataatcactacacacagaagtccctctccctctctccaggcaag

SEQ ID NO: 86 - protein, 451 aa, synthetic construct
EVQLVESGGGLVQPGGSRRVSCAASGFTFSSFGMHWVRQAPGKGLEWVAYISRGSSTIYYADTVKGRFTISRDNAKNSLYLQMNSLRAEDTAVYYCARSGYGSSSYYFDYWGQGTTVTVSSASTKGPSVFPLAPSSKSTSGGTAALGCLVKDYFPEPVTVSWNSGALTSGVHTFPAVLQSSGLYSLSSVVTVPSSSLGTQTYICNVNHKPSNTKVDKKVEPKSCDKTHTCPPCPAPEAAGGPSVFLFPPKPKDTLMISRTPEVTCVVVDVSHEDPEVKFNWYVDGVEVHNAKTKPREEQYNSTYRVVSVLTVLHQDWLNGKEYKCKVSNKALAAPIEKTISKAKGQPREPQVCTLPPSREEMTKNQVSLSCAVKGFYPSDIAVEWESNGQPENNYKTTPPVLDSDGSFFLVSKLTVDKSRWQQGNVFSCSVMHEALHNHYTQKSLSLSPGK

SEQ ID NO: 87 - DNA, 1353 bp, synthetic construct
  source 1..1353: mol_type = other DNA
gaggtgcagctggtcgaatctggaggcggcctggtgcagcccggcggctctagacgggtgtcttgtgccgcttccggcttcacctttagcagcttcggcatgcactgggtgcggcaggcccctggcaagggcctcgagtgggtcgcctacatcagccggggatcttctaccatctactacgccgataccgtgaagggcagattcaccatctcccgggacaacgccaagaatagcctgtacctgcagatgaactccctgagagccgaggacaccgctgtgtactactgcgccagatctggctacggctcttcttcttactatttcgactactggggccaaggcacaaccgtgaccgtttcttccgcctctaccaaaggaccttccgtgtttcctctggctccttcctccaaatccacatctgggggtacagctgccctcggctgcttggtgaaggactacttccccgagcccgtgaccgtgtcctggaactctggcgctctgacctctggagtgcataccttccctgctgtgctgcagtcctccggcctgtactccctgtcctccgtggtgacagtgccttcctctagcctgggcactcagacctatatctgcaacgtgaaccacaaaccttccaacaccaaggtggataagaaggtggaacccaagtcctgcgacaaaacccacacctgtcctccttgccctgccccagaggctgctggcggaccctctgtctttctgttcccacctaagcctaaggacaccctgatgatctctcggacccctgaagtgacctgcgtggtcgtggacgtgtctcacgaggatcctgaggtgaagttcaactggtacgtggacggcgtggaagtgcacaacgctaagaccaagcccagagaagagcagtacaactccacctacagagtggtgtctgtgctgaccgttctgcaccaggactggctgaacggcaaagagtacaagtgcaaggtctccaacaaggctctggccgcacctatcgagaagacaatcagcaaggccaagggccagcctagagaacctcaagtgtgcaccctgcctccaagccgcgaggaaatgaccaagaaccaggtgtccctgtcctgtgccgtgaaaggcttctacccctccgacatcgccgtggaatgggagtccaatggccagcctgagaacaactacaagaccacccctcctgtgctggactccgatggctccttcttcctggtctccaagctgacagtggacaagtctagatggcagcagggcaacgtgttctcgtgctccgtgatgcacgaggccctgcataatcactatacccagaagtctctgtctctgagccctggcaag

SEQ ID NO: 88 - protein, 482 aa, synthetic construct
ELVVTQEPSLTTSPGGTVTLTCRSSTGAVTTSNYANWVQQKPGQAPRGLIGGTNKRAPGTPARFSGSLLGGKAALTITGVQPEDEAEYYCALWYSNLWVFGGGTKLTVLGGGGSGGGGSGGGGSEVQLVESGGGLVQPGGSLRLSCAASGFTFNTYAMNWVRQAPGKGLEWVARIRSKYNNYATYYADSVKDRFTISRDDSKNTAYLQMNNLKTEDTAMYYCVRHGNFGNSYVSWFAYWGQGTLVTVSSGEPKSSDKTHTCPPCPAPEAAGGPSVFLFPPKPKDTLMISRTPEVTCVVVDVSHEDPEVKFNWYVDGVEVHNAKTKPREEQYNSTYRVVSVLTVLHQDWLNGKEYKCKVSNKALAAPIEKTISKAKGQPREPQVYTLPPCREEMTKNQVSLWCLVKGFYPSDIAVEWESNGQPENNYKTTPPVLDSDGSFFLYSKLTVDKSRWQQGNVFSCSVMHEALHNRYTQKSLSLSPGK

SEQ ID NO: 89 - DNA, 1446 bp, synthetic construct
  source 1..1446: mol_type = other DNA
gagctggtggtgacccaagagccttccctgaccacctcccctggtggcacagtgaccctgacatgcagatcctctaccggcgctgtgacaacgtccaattacgccaattgggtccaacagaagcctggccaggcccccagaggcctgatcggaggcaccaacaagagagccccaggcacccctgctcggttctctggctctctgctgggcggcaaggctgccctgaccatcaccggcgtgcagcccgaggacgaggccgagtactactgtgctctgtggtattccaacctgtgggtctttggcggcggcaccaagctgaccgtgctgggaggcggcggctctggcggcggcggcagcggaggcggaggctccgaggtgcagctggtagaatctggcggcggactagtgcagcctggcggcagcctgagactgtcttgcgccgcctccggcttcacctttaacacatacgcgatgaactgggtgcggcaggctcctggcaagggcctggaatgggtggcccggatccggtccaagtacaacaactatgctacctattacgccgactccgtgaaggacagattcaccatctcccgggacgacagcaagaacaccgcctacctgcagatgaacaacctgaagaccgaggataccgccatgtactactgcgtgcggcacggcaacttcggtaattcctacgtctcttggttcgcctactggggccagggaacactggtgaccgtgtccagcggcgagcctaagtcctccgataaaacccacacctgtcctccttgccctgcccctgaagctgctggcggcccctccgtgtttctgttcccccctaagcccaaggacaccctgatgatctccagaacccctgaggtgacatgtgtggtggtggacgtgtcccacgaggaccctgaagtgaagttcaactggtacgtggatggcgtggaagtgcacaacgccaagaccaagccccgcgaggaacagtacaactccacctacagagtggtcagcgttctcaccgtgctgcatcaagactggctgaacggcaaagagtacaagtgcaaggtgtctaacaaggccctggccgctcctatcgagaagaccatctctaaagccaaaggacagccaagggaacctcaggtctacaccctgcctccatgccgggaagagatgaccaagaaccaggtgtctctctggtgcctggtcaagggcttctacccttctgatatcgccgtggagtgggaatccaatggccagcctgagaacaactacaagacaaccccccctgtgctggactccgacggctccttcttcctgtactctaagctgaccgtggacaagtctagatggcagcagggcaacgtgttctcctgctccgtgatgcacgaggctctgcacaacagatacacccagaaatcgctgtctctgagccctggaaag

SEQ ID NO: 90 - protein, 445 aa, synthetic construct
QVQLVQSGAEVKKPGASVKVSCKASGYSFTGYTMNWVRQAPGQGLEWMGLINPYNSDTNYAQKLQGRVTMTTDTSTSTAYMELRSLRSDDTAVYYCARVALRVALDYWGQGTLVTVSSASTKGPSVFPLAPCSRSTSESTAALGCLVKDYFPEPVTVSWNSGALTSGVHTFPAVLQSSGLYSLSSVVTVPSSSLGTKTYTCNVDHKPSNTKVDKRVESKYGPPCPPCPAPEAAGGPSVFLFPPKPKDTLMISRTPEVTCVVVDVSQEDPEVQFNWYVDGVEVHNAKTKPREEQFNSTYRVVSVLTVLHQDWLNGKEYKCKVSNKGLPSSIEKTISKAKGQPREPQVYTLPPSQEEMTKNQVSLTCLVKGFYPSDIAVEWESNGQPENNYKTTPPVLDSDGSFFLYSRLTVDKSRWQEGNVFSCSVMHEALHNHYTQKSLSLSLGK

SEQ ID NO: 91 - protein, 214 aa, synthetic construct
DIQMTQSPSSLSASVGDRVTITCKASQNVATHVGWYQQKPGKAPKRLIYSASYRYSGVPSRFSGSGSGTEFTLTISNLQPEDFATYYCQQYNRYPYTFGQGTKLEIKRTVAAPSVFIFPPSDEQLKSGTASVVCLLNNFYPREAKVQWKVDNALQSGNSQESVTEQDSKDSTYSLSSTLTLSKADYEKHKVYACEVTHQGLSSPVTKSFNRGEC

SEQ ID NO: 92 - protein, 452 aa, synthetic construct
EVQLVESGGGLVQPGGSLRLSCAASGFTFNTYAMNWVRQAPGKGLEWVARIRSKYNNYATYYAASVKGRFTISRDDSKNSLYLQMNSLKTEDTAVYYCARHGNFGNSYVSWFAYWGQGTLVTVSSASTKGPSVFPLAPCSRSTSESTAALGCLVKDYFPEPVTVSWNSGALTSGVHTFPAVLQSSGLYSLSSVVTVPSSSLGTKTYTCNVDHKPSNTKVDKRVESKYGPPCPPCPAPEAAGGPSVFLFPPKPKDTLMISRTPEVTCVVVDVSQEDPEVQFNWYVDGVEVHNAKTKPREEQFNSTYRVVSVLTVLHQDWLNGKEYKCKVSNKGLPSSIEKTISKAKGQPREPQVYTLPPSQEEMTKNQVSLTCLVKGFYPSDIAVEWESNGQPENNYKTTPPVLDSDGSFLLYSKLTVDKSRWQEGNVFSCSVMHEALHNHYTQKSLSLSLGK

SEQ ID NO: 93 - protein, 215 aa, synthetic construct
QTVVTQEPSLTVSPGGTVTLTCRSSTGAVTTSNYANWVQQKPGQAPRGLIGGTNKRAPGTPARFSGSLLGGKAALTLSGVQPEDEAEYYCALWYSNLWVFGGGTKLTVLGQPKAAPSVTLFPPSSEELQANKATLVCLISDFYPGAVTVAWKADSSPVKAGVETTTPSKQSNNKYAASSYLSLTPEQWKSHRSYSCQVTHEGSTVEKTVAPTECS

SEQ ID NO: 94 - protein, 5 aa, synthetic construct
TYAMN

SEQ ID NO: 95 - protein, 19 aa, synthetic construct
RIRSKYNNYATYYADSVKD

SEQ ID NO: 96 - protein, 14 aa, synthetic construct
HGNFGNSYVSWFAY

SEQ ID NO: 97 - protein, 14 aa, synthetic construct
RSSTGAVTTSNYAN

SEQ ID NO: 98 - protein, 7 aa, synthetic construct
GTNKRAP

SEQ ID NO: 99 - protein, 9 aa, synthetic construct
ALWYSNLWV

SEQ ID NO: 100 - protein, 125 aa, synthetic construct
EVQLVESGGGLVQPGGSLRLSCAASGFTFNTYAMNWVRQAPGKGLEWVARIRSKYNNYATYYADSVKDRFTISRDDSKNTAYLQMNNLKTEDTAMYYCVRHGNFGNSYVSWFAYWGQGTLVTVSS

SEQ ID NO: 101 - protein, 109 aa, synthetic construct
ELVVTQEPSLTTSPGGTVTLTCRSSTGAVTTSNYANWVQQKPGQAPRGLIGGTNKRAPGTPARFSGSLLGGKAALTITGVQPEDEAEYYCALWYSNLWVFGGGTKLTVL

SEQ ID NO: 102 - protein, 15 aa, synthetic construct
EPKSCDKTHTCPPCP

SEQ ID NO: 103 - protein, 16 aa, synthetic construct
GEPKSSDKTHTCPPCP

SEQ ID NO: 104 - protein, 5 aa, synthetic construct
GGGGS